European Patent Application EP 4 772 537 A2, published July 8, 2026. Title: METHOD FOR TREATING CANCER USING A BCL-2 INHIBITOR IN CONJUNCTION WITH AN ALPHA-EMITTING RADIOIMMUNOTHERAPEUTIC. Applicant: ACTINIUM PHARMACEUTICALS, INC. Application EP PCT/US2018/029607, filed April 26, 2018. The sequence listing filed with the application follows.

SEQUENCE LISTING (4 sequences)

SEQ ID NO: 1 - DNA, 1952 bp, synthetic construct
  misc_feature 1..1952: note = Description of Artificial Sequence: Synthetic polynucleotide
  source 1..1952: mol_type = other DNA
tctagaccaccatggagaaagacacactcctgctatgggtcctacttctctgggttccaggttccacaggtgacattcagatgacccagtctccgagctctctgtccgcatcagtaggagacagggtcaccatcacatgcagagccagcgaaagtgtcgacaattatggcattagctttatgaactggttccaacagaaacccgggaaggctcctaagcttctgatttacgctgcatccaaccaaggctccggggtaccctctcgcttctcaggcagtggatctgggacagacttcactctcaccatttcatctctgcagcctgatgacttcgcaacctattactgtcagcaaagtaaggaggttccgtggacgttcggtcaagggaccaaggtggagatcaaacgtaagtagaatccaaagtctagaaattctaaactctgagggggtcggatgacgtggccattctttgcctaaagcattgagtttactgcaaggtcagaaaagcatgcaaagccctcagaatggctgcaaagagctccaacaaaacaatttagaactttattaaggaatagggggaagctaggaagaaactcaaaacatcaagattttaaatacgcttcttggtctccttgctataattatctgggataagcatgctgttttctgtctgtccctaacatgctctgtgattatccgcaaacaacacacccaagggcagaactttgttacttaaacaccatcctgtttgcttctttcctcaggaactgtggctgcaccatctgtcttcatcttcccgccatctgatgagcagttgaaatctggaactgcctctgttgtgtgcctgctgaataacttctatcccagagaggccaaagtacagtggaaggtggataacgccctccaatcgggtaactcccaggagagtgtcacagagcaggacagcaaggacagcacctacagcctcagcagcaccctgacgctgagcaaagcagactacgagaaacacaaagtctacgcctgcgaagtcacccatcagggcctgagctcgcccgtcacaaagagcttcaacaggggagagtgttagagggagaagtgcccccacctgctcctcagttccagcctgaccccctcccatcctttggcctctgaccctttttccacaggggacctacccctattgcggtcctccagctcatctttcacctcacccccctcctcctccttggctttaattatgctaatgttggaggagaatgaataaataaagtgaatctttgcacctgtggtttctctctttcctcatttaataattattatctgttgttttaccaactactcaatttctcttataagggactaaatatgtagtcatcctaaggcgcataaccatttataaaaatcatccttcattctattttaccctatcatcctctgcaagacagtcctccctcaaacccacaagccttctgtcctcacagtcccctgggccatggtaggagagacttgcttccttgttttcccctcctcagcaagccctcatagtcctttttaagggtgacaggtcttacagtcatatatcctttgattcaattccctgagaatcaaccaaagcaaatttttcaaaagaagaaacctgctataaagagaatcattcattgcaacatgatataaaataacaacacaataaaagcaattaaataaacaaacaatagggaaatgtttaagttcatcatggtacttagacttaatggaatgtcatgccttatttacatttttaaacaggtactgagggactcctgtctgccaagggccgtattgagtactttccacaacctaatttaatccacactatactgtgagattaaaaacattcattaaaatgttgcaaaggttctataaagctgagagacaaatatattctataactcagcaatcccacttctaggatcc

SEQ ID NO: 2 - protein, 238 aa, synthetic construct
  REGION 1..238: note = Description of Artificial Sequence: Synthetic polypeptide
MEKDTLLLWVLLLWVPGSTGDIQMTQSPSSLSASVGDRVTITCRASESVDNYGISFMNWFQQKPGKAPKLLIYAASNQGSGVPSRFSGSGSGTDFTLTISSLQPDDFATYYCQQSKEVPWTFGQGTKVEIKRTVAAPSVFIFPPSDEQLKSGTASVVCLLNNFYPREAKVQWKVDNALQSGNSQESVTEQDSKDSTYSLSSTLTLSKADYEKHKVYACEVTHQGLSSPVTKSFNRGEC

SEQ ID NO: 3 - DNA, 3246 bp, synthetic construct
  misc_feature 1..3246: note = Description of Artificial Sequence: Synthetic polynucleotide
  source 1..3246: mol_type = other DNA
tctagaccaccatgggatggagctggatctttctcttcctcctgtcaggaactgctggcgtccactctcaggttcagctggtgcagtctggagctgaggtgaagaagcctgggagctcagtgaaggtttcctgcaaagcttctggctacaccttcactgactacaacatgcactgggtgaggcaggctcctggccaaggcctggaatggattggatatatttatccttacaatggtggtaccggctacaaccagaagttcaagagcaaggccacaattacagcagacgagagtactaacacagcctacatggaactctccagcctgaggtctgaggacactgcagtctattactgcgcaagagggcgccccgctatggactactggggccaagggactctggtcactgtctcttcaggtaagaatggcctctagaccaccatgggatggagctttctggggcaggccaggcctgaccttggctttggggcagggagggggctaaggtgaggcaggtggcgccagccaggtgcacacccaatgcccatgagcccagacactggacgctgaacctcgcggacagttaagaacccaggggcctctgcgccctgggcccagctctgtcccacaccgcggtcacatggcaccacctctcttgcagcctccaccaagggcccatcggtcttccccctggcaccctcctccaagagcacctctgggggcacagcggccctgggctgcctggtcaaggactacttccccgaaccggtgacggtgtcgtggaactcaggcgccctgaccagcggcgtgcacaccttcccggctgtcctacagtcctcaggactctactccctcagcagcgtggtgaccgtgccctccagcagcttgggcacccagacctacatctgcaacgtgaatcacaagcccagcaacaccaaggtggacaagaaagttggtgagaggccagcacagggagggagggtgtctgctggaagccaggctcagcgctcctgcctggacgcatcccggctatgcagccccagtccagggcagcaaggcaggccccgtctgcctcttcacccggaggcctctgcccgccccactcatgctcagggagagggtcttctggctttttccccaggctctgggcaggcacaggctaggtgcccctaacccaggccctgcacacaaaggggcaggtgctgggctcagacctgccaagagccatatccgggaggaccctgcccctgacctaagcccaccccaaaggccaaactctccactccctcagctcggacaccttctctcctcccagattccagtaactcccaatcttctctctgcagagcccaaatcttgtgacaaaactcacacatgcccaccgtgcccaggtaagccagcccaggcctcgccctccagctcaaggcgggacaggtgccctagagtagcctgcatccagggacaggccccagccgggtgctgacacgtccacctccatctcttcctcagcacctgaactcctggggggaccgtcagtcttcctcttccccccaaaacccaaggacaccctcatgatctcccggacccctgaggtcacatgcgtggtggtggacgtgagccacgaagaccctgaggtcaagttcaactggtacgtggacggcgtggaggtgcataatgccaagacaaagccgcgggaggagcagtacaacagcacgtaccgtgtggtcagcgtcctcaccgtcctgcaccaggactggctgaatggcaaggagtacaagtgcaaggtctccaacaaagccctcccagcccccatcgagaaaaccatctccaaagccaaaggtgggacccgtggggtgcgagggccacatggacagaggccggctcggcccaccctctgccctgagagtgaccgctgtaccaacctctgtccctacagggcagccccgagaaccacaggtgtacaccctgcccccatcccgggatgagctgaccaagaaccaggtcagcctgacctgcctggtcaaaggcttctatcccagcgacatcgccgtggagtgggagagcaatgggcagccggagaacaactacaagaccacgcctcccgtgctggactccgacggctccttcttcctctacagcaagctcaccgtggacaagagcaggtggcagcaggggaacgtcttctcatgctccgtgatgcatgaggctctgcacaaccactacacgcagaagagcctctccctgtctccgggtaaatgagtgcgacggccggcaagcccccgctccccgggctctcgcggtcgcacgaggatgcttggcacgtaccccctgtacatacttcccgggcgcccagcatggaaataaagcacccagcgctgccctgggcccctgcgagactgtgatggttctttccacgggtcaggccgagtctgaggcctgagtggcatgagggaggcagagcgggtcccactgtccccacactggcccaggctgtgcaggtgtgcctgggccgcctagggtggggctcagccaggggctgccctcggcagggtgggggatttgccagcgtggccctccctccagcagcacctgccctgggctgggccacgggaagccctaggagcccctggggacagacacacagcccctgcctctgtaggagactgtcctgttctgtgagcgccctgtcctccgacctccatgcccactcgggggcatgcctagtccatgtgcgtagggacaggccctccctcacccatctacccccacggcactaacccctggctgccctgcccagcctcgcacccgcatggggacacaaccgactccggggacatgcactctcgggccctgtggagggactggtgcagatgcccacacacacactcagcccagacccgttcaacaaaccccgcactgaggttggccggccacacggccaccacacacacacgtgcacgcctcacacacggagcctcacccgggcgaactgcacagcacccagaccagagcaaggtcctcgcacacgtgaacactcctcggacacaggcccccacgagccccacgcggcacctcaaggcccacgagcctctcggcagcttctccacatgctgacctgctcagacaaacccagccctcctctcacaagggtgcccctgcagccgccacacacacacaggggatcacacaccacgtcacgtccctggccctggcccacttcccagtgccgcccttccctgcaggatcc

SEQ ID NO: 4 - protein, 465 aa, synthetic construct
  REGION 1..465: note = Description of Artificial Sequence: Synthetic polypeptide
MGWSWIFLFLLSGTAGVHSQVQLVQSGAEVKKPGSSVKVSCKASGYTFTDYNMHWVRQAPGQGLEWIGYIYPYNGGTGYNQKFKSKATITADESTNTAYMELSSLRSEDTAVYYCARGRPAMDYWGQGTLVTVSSASTKGPSVFPLAPSSKSTSGGTAALGCLVKDYFPEPVTVSWNSGALTSGVHTFPAVLQSSGLYSLSSVVTVPSSSLGTQTYICNVNHKPSNTKVDKKVEPKSCDKTHTCPPCPAPELLGGPSVFLFPPKPKDTLMISRTPEVTCVVVDVSHEDPEVKFNWYVDGVEVHNAKTKPREEQYNSTYRVVSVLTVLHQDWLNGKEYKCKVSNKALPAPIEKTISKAKGQPREPQVYTLPPSRDELTKNQVSLTCLVKGFYPSDIAVEWESNGQPENNYKTTPPVLDSDGSFFLYSKLTVDKSRWQQGNVFSCSVMHEALHNHYTQKSLSLSPGK